European Patent Specification EP 4 321 536 B1, published April 1, 2026. Title: BISPECIFIC ANTIBODIES AND USES OF THE SAME THEREOF. Applicant: Hefei TG ImmunoPharma Co., Ltd. The sequence listing filed with the application follows.

SEQUENCE LISTING (88 sequences)

SEQ ID NO: 1 - protein, 11 aa, Artificial Sequence
  1
RASQDIRNYLN

SEQ ID NO: 2 - protein, 7 aa, Artificial Sequence
  2
YTSRLES

SEQ ID NO: 3 - protein, 9 aa, Artificial Sequence
  3
QQGNTLPWT

SEQ ID NO: 4 - protein, 5 aa, Artificial Sequence
  4
GYTMN

SEQ ID NO: 5 - protein, 17 aa, Artificial Sequence
  5
LINPYKGVSTYNQKFKD

SEQ ID NO: 6 - protein, 13 aa, Artificial Sequence
  6
SGYYGDSDWYFDV

SEQ ID NO: 7 - protein, 15 aa, Artificial Sequence
  7
KASQSVDYDGDSYMN

SEQ ID NO: 8 - protein, 7 aa, Artificial Sequence
  8
AASTLHS

SEQ ID NO: 9 - protein, 9 aa, Artificial Sequence
  9
QQSKEDPRT

SEQ ID NO: 10 - protein, 5 aa, Artificial Sequence
  10
DYNMD

SEQ ID NO: 11 - protein, 17 aa, Artificial Sequence
  11
DINPNNGGTLYNQKFRG

SEQ ID NO: 12 - protein, 11 aa, Artificial Sequence
  12
SEVFYGNYADY

SEQ ID NO: 13 - protein, 108 aa, Artificial Sequence
  13
MDIQMTQSPSSLSASVGDRVTITCRASQDIRNYLNWYQQKPGKAPKLLIYYTSRLESGVPSRFSGSGSGTDYTLTISSLQPEDFATYYCQQGNTLPWTFGQGTKVEIK

SEQ ID NO: 14 - protein, 122 aa, Artificial Sequence [sequence omitted]

SEQ ID NO: 15 - protein, 111 aa, Artificial Sequence
  15
DIVLTQSPVSLAVPLGQRATISCKASQSVDYDGDSYMNWYQQKPGQPPKLLIYAASTLHSGIPVRFSGSGSGTDFTLNIHPVEEEDAASYYCQQSKEDPRTFGGGTKLEIK

SEQ ID NO: 16 - protein, 111 aa, Artificial Sequence
  16
DIVLTQSPDSLAVSLGERATINCKASQSVDYDGDSYMNWYQQKPGQPPKLLIYAASTLHSGVPDRFSGSGSGTDFTLTISSLQAEDVAVYYCQQSKEDPRTFGQGTKLEIK

SEQ ID NO: 17 - protein, 111 aa, Artificial Sequence
  17
DIVLTQSPDSLAVSLGERATINCKASQSVDYDGDSYMNWYQQKPGQPPKLLIYAASTLHSGIPDRFSGSGSGTDFTLTISSLQAEDVAVYYCQQSKEDPRTFGQGTKLEIK

SEQ ID NO: 18 - protein, 111 aa, Artificial Sequence
  18
DIVLTQSPVSLAVPLGQRATISCKASQSVDYDADSYMNWYQQKPGQPPKLLIYAASTLHSGIPVRFSGSGSGTDFTLNIHPVEEEDAASYYCQQSKEDPRTFGGGTKLEIK

SEQ ID NO: 19 - protein, 111 aa, Artificial Sequence
  19
DIVLTQTPLSLSVTPGQPASISCKASQSVDYDGDSYMNWYLQKPGQPPQLLIYAASTLHSGVPDRFSGSGSGTDFTLKISRVEAEDVGVYYCQQSKEDPRTFGQGTKLEIK

SEQ ID NO: 20 - protein, 111 aa, Artificial Sequence
  20
DIVLTQTPLSLSVTPGQPASISCKASQSVDYDGDSYMNWYLQKPGQPPQLLIYAASTLHSGIPDRFSGSGSGTDFTLKISRVEAEDVGVYYCQQSKEDPRTFGQGTKLEIK

SEQ ID NO: 21 - protein, 120 aa, Artificial Sequence
  21
EVLLQQSGPEVVKPGASVKITCKASGYTFTDYNMDWVKQSHGKSLEWIGDINPNNGGTLYNQKFRGRVTLIVDKSSSTAYMELRSLTSDDTAVYYCARSEVFYGNYADYWGQGTTLTVSS

SEQ ID NO: 22 - protein, 120 aa, Artificial Sequence
  22
EVQLVQSGAEVKKPGASVKVSCKASGYTFTDYNMDWVRQAPGQGLEWMGDINPNNGGTLYNQKFRGRVTMTVDTSISTAYMELSRLRSDDTAVYYCARSEVFYGNYADYWGQGTTVTVSS

SEQ ID NO: 23 - protein, 120 aa, Artificial Sequence
  23
EVQLVQSGAEVKKPGASVKVSCKASGYTFTDYNMDWVRQAPGQGLEWIGDINPNNGGTLYNQKFRGRVTLTVDTSISTAYMELSRLRSDDTAVYYCARSEVFYGNYADYWGQGTTVTVSS

SEQ ID NO: 24 - protein, 120 aa, Artificial Sequence
  24
EVQLVQSGAEVKKPGASVKVSCKASGYTFTDYNMDWVRQAPGQGLEWIGDINPNNGGTLYNQKFRGRVTLTVDKSISTAYMELSRLRSDDTAVYYCARSEVFYGNYADYWGQGTTVTVSS

SEQ ID NO: 25 - protein, 120 aa, Artificial Sequence
  25
EVQLVQSGAEVKKPGASVKVSCKASGYTFTDYNMDWVRQAPGKGLEWIGDINPNNGGTLYNQKFRGRVTLTVDKSISTAYMELSRLRSDDTAVYYCARSEVFYGNYADYWGQGTTVTVSS

SEQ ID NO: 26 - protein, 120 aa, Artificial Sequence
  26
EVLLQQSGPEVVKPGASVKITCKASGYTFTDYNMDWVKQSHGKSLEWIGDINPNNAGTLYNQKFRGRVTLIVDKSSSTAYMELRSLTSDDTAVYYCARSEVFYGNYADYWGQGTTLTVSS

SEQ ID NO: 27 - protein, 245 aa, Artificial Sequence
  27
MDIQMTQSPSSLSASVGDRVTITCRASQDIRNYLNWYQQKPGKAPKLLIYYTSRLESGVPSRFSGSGSGTDYTLTISSLQPEDFATYYCQQGNTLPWTFGQGTKVEIKGGGGSGGGGSGGGGSEVQLVESGGGLVQPGGSLRLSCAASGYSFTGYTMNWVRQAPGKGLEWVALINPYKGVSTYNQKFKDRFTISVDKSKNTAYLQMNSLRAEDTAVYYCARSGYYGDSDWYFDVWGQGTLVTVSS

SEQ ID NO: 28 - protein, 246 aa, Artificial Sequence
  28
DIVLTQSPDSLAVSLGERATINCKASQSVDYDGDSYMNWYQQKPGQPPKLLIYAASTLHSGVPDRFSGSGSGTDFTLTISSLQAEDVAVYYCQQSKEDPRTFGQGTKLEIKGGGGSGGGGSGGGGSEVQLVQSGAEVKKPGASVKVSCKASGYTFTDYNMDWVRQAPGQGLEWMGDINPNNGGTLYNQKFRGRVTMTVDTSISTAYMELSRLRSDDTAVYYCARSEVFYGNYADYWGQGTTVTVSS

SEQ ID NO: 29 - protein, 246 aa, Artificial Sequence
  29
DIVLTQSPDSLAVSLGERATINCKASQSVDYDGDSYMNWYQQKPGQPPKLLIYAASTLHSGVPDRFSGSGSGTDFTLTISSLQAEDVAVYYCQQSKEDPRTFGQGTKLEIKGGGGSGGGGSGGGGSEVQLVQSGAEVKKPGASVKVSCKASGYTFTDYNMDWVRQAPGQGLEWIGDINPNNGGTLYNQKFRGRVTLTVDTSISTAYMELSRLRSDDTAVYYCARSEVFYGNYADYWGQGTTVTVSS

SEQ ID NO: 30 - protein, 246 aa, Artificial Sequence
  30
DIVLTQSPDSLAVSLGERATINCKASQSVDYDGDSYMNWYQQKPGQPPKLLIYAASTLHSGVPDRFSGSGSGTDFTLTISSLQAEDVAVYYCQQSKEDPRTFGQGTKLEIKGGGGSGGGGSGGGGSEVQLVQSGAEVKKPGASVKVSCKASGYTFTDYNMDWVRQAPGQGLEWIGDINPNNGGTLYNQKFRGRVTLTVDKSISTAYMELSRLRSDDTAVYYCARSEVFYGNYADYWGQGTTVTVSS

SEQ ID NO: 31 - protein, 246 aa, Artificial Sequence
  31
DIVLTQSPDSLAVSLGERATINCKASQSVDYDGDSYMNWYQQKPGQPPKLLIYAASTLHSGVPDRFSGSGSGTDFTLTISSLQAEDVAVYYCQQSKEDPRTFGQGTKLEIKGGGGSGGGGSGGGGSEVQLVQSGAEVKKPGASVKVSCKASGYTFTDYNMDWVRQAPGKGLEWIGDINPNNGGTLYNQKFRGRVTLTVDKSISTAYMELSRLRSDDTAVYYCARSEVFYGNYADYWGQGTTVTVSS

SEQ ID NO: 32 - protein, 246 aa, Artificial Sequence
  32
DIVLTQSPDSLAVSLGERATINCKASQSVDYDGDSYMNWYQQKPGQPPKLLIYAASTLHSGIPDRFSGSGSGTDFTLTISSLQAEDVAVYYCQQSKEDPRTFGQGTKLEIKGGGGSGGGGSGGGGSEVQLVQSGAEVKKPGASVKVSCKASGYTFTDYNMDWVRQAPGQGLEWMGDINPNNGGTLYNQKFRGRVTMTVDTSISTAYMELSRLRSDDTAVYYCARSEVFYGNYADYWGQGTTVTVSS

SEQ ID NO: 33 - protein, 246 aa, Artificial Sequence
  33
DIVLTQSPDSLAVSLGERATINCKASQSVDYDGDSYMNWYQQKPGQPPKLLIYAASTLHSGIPDRFSGSGSGTDFTLTISSLQAEDVAVYYCQQSKEDPRTFGQGTKLEIKGGGGSGGGGSGGGGSEVQLVQSGAEVKKPGASVKVSCKASGYTFTDYNMDWVRQAPGQGLEWIGDINPNNGGTLYNQKFRGRVTLTVDTSISTAYMELSRLRSDDTAVYYCARSEVFYGNYADYWGQGTTVTVSS

SEQ ID NO: 34 - protein, 246 aa, Artificial Sequence
  34
DIVLTQSPDSLAVSLGERATINCKASQSVDYDGDSYMNWYQQKPGQPPKLLIYAASTLHSGIPDRFSGSGSGTDFTLTISSLQAEDVAVYYCQQSKEDPRTFGQGTKLEIKGGGGSGGGGSGGGGSEVQLVQSGAEVKKPGASVKVSCKASGYTFTDYNMDWVRQAPGQGLEWIGDINPNNGGTLYNQKFRGRVTLTVDKSISTAYMELSRLRSDDTAVYYCARSEVFYGNYADYWGQGTTVTVSS

SEQ ID NO: 35 - protein, 246 aa, Artificial Sequence
  35
DIVLTQSPDSLAVSLGERATINCKASQSVDYDGDSYMNWYQQKPGQPPKLLIYAASTLHSGIPDRFSGSGSGTDFTLTISSLQAEDVAVYYCQQSKEDPRTFGQGTKLEIKGGGGSGGGGSGGGGSEVQLVQSGAEVKKPGASVKVSCKASGYTFTDYNMDWVRQAPGKGLEWIGDINPNNGGTLYNQKFRGRVTLTVDKSISTAYMELSRLRSDDTAVYYCARSEVFYGNYADYWGQGTTVTVSS

SEQ ID NO: 36 - protein, 246 aa, Artificial Sequence
  36
DIVLTQTPLSLSVTPGQPASISCKASQSVDYDGDSYMNWYLQKPGQPPQLLIYAASTLHSGVPDRFSGSGSGTDFTLKISRVEAEDVGVYYCQQSKEDPRTFGQGTKLEIKGGGGSGGGGSGGGGSEVQLVQSGAEVKKPGASVKVSCKASGYTFTDYNMDWVRQAPGQGLEWMGDINPNNGGTLYNQKFRGRVTMTVDTSISTAYMELSRLRSDDTAVYYCARSEVFYGNYADYWGQGTTVTVSS

SEQ ID NO: 37 - protein, 246 aa, Artificial Sequence
  37
DIVLTQTPLSLSVTPGQPASISCKASQSVDYDGDSYMNWYLQKPGQPPQLLIYAASTLHSGVPDRFSGSGSGTDFTLKISRVEAEDVGVYYCQQSKEDPRTFGQGTKLEIKGGGGSGGGGSGGGGSEVQLVQSGAEVKKPGASVKVSCKASGYTFTDYNMDWVRQAPGQGLEWIGDINPNNGGTLYNQKFRGRVTLTVDTSISTAYMELSRLRSDDTAVYYCARSEVFYGNYADYWGQGTTVTVSS

SEQ ID NO: 38 - protein, 246 aa, Artificial Sequence
  38
DIVLTQTPLSLSVTPGQPASISCKASQSVDYDGDSYMNWYLQKPGQPPQLLIYAASTLHSGVPDRFSGSGSGTDFTLKISRVEAEDVGVYYCQQSKEDPRTFGQGTKLEIKGGGGSGGGGSGGGGSEVQLVQSGAEVKKPGASVKVSCKASGYTFTDYNMDWVRQAPGQGLEWIGDINPNNGGTLYNQKFRGRVTLTVDKSISTAYMELSRLRSDDTAVYYCARSEVFYGNYADYWGQGTTVTVSS

SEQ ID NO: 39 - protein, 246 aa, Artificial Sequence
  39
DIVLTQTPLSLSVTPGQPASISCKASQSVDYDGDSYMNWYLQKPGQPPQLLIYAASTLHSGVPDRFSGSGSGTDFTLKISRVEAEDVGVYYCQQSKEDPRTFGQGTKLEIKGGGGSGGGGSGGGGSEVQLVQSGAEVKKPGASVKVSCKASGYTFTDYNMDWVRQAPGKGLEWIGDINPNNGGTLYNQKFRGRVTLTVDKSISTAYMELSRLRSDDTAVYYCARSEVFYGNYADYWGQGTTVTVSS

SEQ ID NO: 40 - protein, 246 aa, Artificial Sequence
  40
DIVLTQTPLSLSVTPGQPASISCKASQSVDYDGDSYMNWYLQKPGQPPQLLIYAASTLHSGIPDRFSGSGSGTDFTLKISRVEAEDVGVYYCQQSKEDPRTFGQGTKLEIKGGGGSGGGGSGGGGSEVQLVQSGAEVKKPGASVKVSCKASGYTFTDYNMDWVRQAPGQGLEWMGDINPNNGGTLYNQKFRGRVTMTVDTSISTAYMELSRLRSDDTAVYYCARSEVFYGNYADYWGQGTTVTVSS

SEQ ID NO: 41 - protein, 246 aa, Artificial Sequence
  41
DIVLTQTPLSLSVTPGQPASISCKASQSVDYDGDSYMNWYLQKPGQPPQLLIYAASTLHSGIPDRFSGSGSGTDFTLKISRVEAEDVGVYYCQQSKEDPRTFGQGTKLEIKGGGGSGGGGSGGGGSEVQLVQSGAEVKKPGASVKVSCKASGYTFTDYNMDWVRQAPGQGLEWIGDINPNNGGTLYNQKFRGRVTLTVDTSISTAYMELSRLRSDDTAVYYCARSEVFYGNYADYWGQGTTVTVSS

SEQ ID NO: 42 - protein, 246 aa, Artificial Sequence
  42
DIVLTQTPLSLSVTPGQPASISCKASQSVDYDGDSYMNWYLQKPGQPPQLLIYAASTLHSGIPDRFSGSGSGTDFTLKISRVEAEDVGVYYCQQSKEDPRTFGQGTKLEIKGGGGSGGGGSGGGGSEVQLVQSGAEVKKPGASVKVSCKASGYTFTDYNMDWVRQAPGQGLEWIGDINPNNGGTLYNQKFRGRVTLTVDKSISTAYMELSRLRSDDTAVYYCARSEVFYGNYADYWGQGTTVTVSS

SEQ ID NO: 43 - protein, 246 aa, Artificial Sequence
  43
DIVLTQTPLSLSVTPGQPASISCKASQSVDYDGDSYMNWYLQKPGQPPQLLIYAASTLHSGIPDRFSGSGSGTDFTLKISRVEAEDVGVYYCQQSKEDPRTFGQGTKLEIKGGGGSGGGGSGGGGSEVQLVQSGAEVKKPGASVKVSCKASGYTFTDYNMDWVRQAPGKGLEWIGDINPNNGGTLYNQKFRGRVTLTVDKSISTAYMELSRLRSDDTAVYYCARSEVFYGNYADYWGQGTTVTVSS

SEQ ID NO: 44 - protein, 246 aa, Artificial Sequence
  44
DIVLTQSPVSLAVPLGQRATISCKASQSVDYDGDSYMNWYQQKPGQPPKLLIYAASTLHSGIPVRFSGSGSGTDFTLNIHPVEEEDAASYYCQQSKEDPRTFGGGTKLEIKGGGGSGGGGSGGGGSEVLLQQSGPEVVKPGASVKITCKASGYTFTDYNMDWVKQSHGKSLEWIGDINPNNAGTLYNQKFRGRVTLIVDKSSSTAYMELRSLTSDDTAVYYCARSEVFYGNYADYWGQGTTLTVSS

SEQ ID NO: 45 - protein, 246 aa, Artificial Sequence
  45
DIVLTQSPVSLAVPLGQRATISCKASQSVDYDADSYMNWYQQKPGQPPKLLIYAASTLHSGIPVRFSGSGSGTDFTLNIHPVEEEDAASYYCQQSKEDPRTFGGGTKLEIKGGGGSGGGGSGGGGSEVLLQQSGPEVVKPGASVKITCKASGYTFTDYNMDWVKQSHGKSLEWIGDINPNNGGTLYNQKFRGRVTLIVDKSSSTAYMELRSLTSDDTAVYYCARSEVFYGNYADYWGQGTTLTVSS

SEQ ID NO: 46 - protein, 15 aa, Artificial Sequence
  46
GGGGSGGGGSGGGGS

SEQ ID NO: 47 - protein, 232 aa, Artificial Sequence
  47
EPKSCDKTHTCPPCPAPEAAGGPSVFLFPPKPKDTLMISRTPEVTCVVVDVSHEDPEVKFNWYVDGVEVHNAKTKPREEQYNSTYRVVSVLTVLHQDWLNGKEYKCKVSNKALPAPIEKTISKAKGQPREPQVYTLPPCRDELTKNQVSLWCLVKGFYPSDIAVEWESNGQPENNYKTTPPVLDSDGSFFLYSKLTVDKSRWQQGNVFSCSVMHEALHNHYTQKSLSLSPGK

SEQ ID NO: 48 - protein, 232 aa, Artificial Sequence
  48
EPKSCDKTHTCPPCPAPEAAGGPSVFLFPPKPKDTLMISRTPEVTCVVVDVSHEDPEVKFNWYVDGVEVHNAKTKPREEQYNSTYRVVSVLTVLHQDWLNGKEYKCKVSNKALPAPIEKTISKAKGQPREPQVCTLPPSRDELTKNQVSLSCAVKGFYPSDIAVEWESNGQPENNYKTTPPVLDSDGSFFLVSKLTVDKSRWQQGNVFSCSVMHEALHNHYTQKSLSLSPGK

SEQ ID NO: 49 - protein, 477 aa, Artificial Sequence
  49
MDIQMTQSPSSLSASVGDRVTITCRASQDIRNYLNWYQQKPGKAPKLLIYYTSRLESGVPSRFSGSGSGTDYTLTISSLQPEDFATYYCQQGNTLPWTFGQGTKVEIKGGGGSGGGGSGGGGSEVQLVESGGGLVQPGGSLRLSCAASGYSFTGYTMNWVRQAPGKGLEWVALINPYKGVSTYNQKFKDRFTISVDKSKNTAYLQMNSLRAEDTAVYYCARSGYYGDSDWYFDVWGQGTLVTVSSEPKSCDKTHTCPPCPAPEAAGGPSVFLFPPKPKDTLMISRTPEVTCVVVDVSHEDPEVKFNWYVDGVEVHNAKTKPREEQYNSTYRVVSVLTVLHQDWLNGKEYKCKVSNKALPAPIEKTISKAKGQPREPQVYTLPPCRDELTKNQVSLWCLVKGFYPSDIAVEWESNGQPENNYKTTPPVLDSDGSFFLYSKLTVDKSRWQQGNVFSCSVMHEALHNHYTQKSLSLSPGK

SEQ ID NO: 50 - protein, 478 aa, Artificial Sequence
  50
DIVLTQSPDSLAVSLGERATINCKASQSVDYDGDSYMNWYQQKPGQPPKLLIYAASTLHSGVPDRFSGSGSGTDFTLTISSLQAEDVAVYYCQQSKEDPRTFGQGTKLEIKGGGGSGGGGSGGGGSEVQLVQSGAEVKKPGASVKVSCKASGYTFTDYNMDWVRQAPGQGLEWMGDINPNNGGTLYNQKFRGRVTMTVDTSISTAYMELSRLRSDDTAVYYCARSEVFYGNYADYWGQGTTVTVSSEPKSCDKTHTCPPCPAPEAAGGPSVFLFPPKPKDTLMISRTPEVTCVVVDVSHEDPEVKFNWYVDGVEVHNAKTKPREEQYNSTYRVVSVLTVLHQDWLNGKEYKCKVSNKALPAPIEKTISKAKGQPREPQVCTLPPSRDELTKNQVSLSCAVKGFYPSDIAVEWESNGQPENNYKTTPPVLDSDGSFFLVSKLTVDKSRWQQGNVFSCSVMHEALHNHYTQKSLSLSPGK

SEQ ID NO: 51 - protein, 478 aa, Artificial Sequence
  51
DIVLTQSPDSLAVSLGERATINCKASQSVDYDGDSYMNWYQQKPGQPPKLLIYAASTLHSGVPDRFSGSGSGTDFTLTISSLQAEDVAVYYCQQSKEDPRTFGQGTKLEIKGGGGSGGGGSGGGGSEVQLVQSGAEVKKPGASVKVSCKASGYTFTDYNMDWVRQAPGQGLEWIGDINPNNGGTLYNQKFRGRVTLTVDTSISTAYMELSRLRSDDTAVYYCARSEVFYGNYADYWGQGTTVTVSSEPKSCDKTHTCPPCPAPEAAGGPSVFLFPPKPKDTLMISRTPEVTCVVVDVSHEDPEVKFNWYVDGVEVHNAKTKPREEQYNSTYRVVSVLTVLHQDWLNGKEYKCKVSNKALPAPIEKTISKAKGQPREPQVCTLPPSRDELTKNQVSLSCAVKGFYPSDIAVEWESNGQPENNYKTTPPVLDSDGSFFLVSKLTVDKSRWQQGNVFSCSVMHEALHNHYTQKSLSLSPGK

SEQ ID NO: 52 - protein, 478 aa, Artificial Sequence
  52
DIVLTQSPDSLAVSLGERATINCKASQSVDYDGDSYMNWYQQKPGQPPKLLIYAASTLHSGVPDRFSGSGSGTDFTLTISSLQAEDVAVYYCQQSKEDPRTFGQGTKLEIKGGGGSGGGGSGGGGSEVQLVQSGAEVKKPGASVKVSCKASGYTFTDYNMDWVRQAPGQGLEWIGDINPNNGGTLYNQKFRGRVTLTVDKSISTAYMELSRLRSDDTAVYYCARSEVFYGNYADYWGQGTTVTVSSEPKSCDKTHTCPPCPAPEAAGGPSVFLFPPKPKDTLMISRTPEVTCVVVDVSHEDPEVKFNWYVDGVEVHNAKTKPREEQYNSTYRVVSVLTVLHQDWLNGKEYKCKVSNKALPAPIEKTISKAKGQPREPQVCTLPPSRDELTKNQVSLSCAVKGFYPSDIAVEWESNGQPENNYKTTPPVLDSDGSFFLVSKLTVDKSRWQQGNVFSCSVMHEALHNHYTQKSLSLSPGK

SEQ ID NO: 53 - protein, 478 aa, Artificial Sequence
  53
DIVLTQSPDSLAVSLGERATINCKASQSVDYDGDSYMNWYQQKPGQPPKLLIYAASTLHSGVPDRFSGSGSGTDFTLTISSLQAEDVAVYYCQQSKEDPRTFGQGTKLEIKGGGGSGGGGSGGGGSEVQLVQSGAEVKKPGASVKVSCKASGYTFTDYNMDWVRQAPGKGLEWIGDINPNNGGTLYNQKFRGRVTLTVDKSISTAYMELSRLRSDDTAVYYCARSEVFYGNYADYWGQGTTVTVSSEPKSCDKTHTCPPCPAPEAAGGPSVFLFPPKPKDTLMISRTPEVTCVVVDVSHEDPEVKFNWYVDGVEVHNAKTKPREEQYNSTYRVVSVLTVLHQDWLNGKEYKCKVSNKALPAPIEKTISKAKGQPREPQVCTLPPSRDELTKNQVSLSCAVKGFYPSDIAVEWESNGQPENNYKTTPPVLDSDGSFFLVSKLTVDKSRWQQGNVFSCSVMHEALHNHYTQKSLSLSPGK

SEQ ID NO: 54 - protein, 478 aa, Artificial Sequence
  54
DIVLTQSPDSLAVSLGERATINCKASQSVDYDGDSYMNWYQQKPGQPPKLLIYAASTLHSGIPDRFSGSGSGTDFTLTISSLQAEDVAVYYCQQSKEDPRTFGQGTKLEIKGGGGSGGGGSGGGGSEVQLVQSGAEVKKPGASVKVSCKASGYTFTDYNMDWVRQAPGQGLEWMGDINPNNGGTLYNQKFRGRVTMTVDTSISTAYMELSRLRSDDTAVYYCARSEVFYGNYADYWGQGTTVTVSSEPKSCDKTHTCPPCPAPEAAGGPSVFLFPPKPKDTLMISRTPEVTCVVVDVSHEDPEVKFNWYVDGVEVHNAKTKPREEQYNSTYRVVSVLTVLHQDWLNGKEYKCKVSNKALPAPIEKTISKAKGQPREPQVCTLPPSRDELTKNQVSLSCAVKGFYPSDIAVEWESNGQPENNYKTTPPVLDSDGSFFLVSKLTVDKSRWQQGNVFSCSVMHEALHNHYTQKSLSLSPGK

SEQ ID NO: 55 - protein, 478 aa, Artificial Sequence
  55
DIVLTQSPDSLAVSLGERATINCKASQSVDYDGDSYMNWYQQKPGQPPKLLIYAASTLHSGIPDRFSGSGSGTDFTLTISSLQAEDVAVYYCQQSKEDPRTFGQGTKLEIKGGGGSGGGGSGGGGSEVQLVQSGAEVKKPGASVKVSCKASGYTFTDYNMDWVRQAPGQGLEWIGDINPNNGGTLYNQKFRGRVTLTVDTSISTAYMELSRLRSDDTAVYYCARSEVFYGNYADYWGQGTTVTVSSEPKSCDKTHTCPPCPAPEAAGGPSVFLFPPKPKDTLMISRTPEVTCVVVDVSHEDPEVKFNWYVDGVEVHNAKTKPREEQYNSTYRVVSVLTVLHQDWLNGKEYKCKVSNKALPAPIEKTISKAKGQPREPQVCTLPPSRDELTKNQVSLSCAVKGFYPSDIAVEWESNGQPENNYKTTPPVLDSDGSFFLVSKLTVDKSRWQQGNVFSCSVMHEALHNHYTQKSLSLSPGK

SEQ ID NO: 56 - protein, 478 aa, Artificial Sequence
  56
DIVLTQSPDSLAVSLGERATINCKASQSVDYDGDSYMNWYQQKPGQPPKLLIYAASTLHSGIPDRFSGSGSGTDFTLTISSLQAEDVAVYYCQQSKEDPRTFGQGTKLEIKGGGGSGGGGSGGGGSEVQLVQSGAEVKKPGASVKVSCKASGYTFTDYNMDWVRQAPGQGLEWIGDINPNNGGTLYNQKFRGRVTLTVDKSISTAYMELSRLRSDDTAVYYCARSEVFYGNYADYWGQGTTVTVSSEPKSCDKTHTCPPCPAPEAAGGPSVFLFPPKPKDTLMISRTPEVTCVVVDVSHEDPEVKFNWYVDGVEVHNAKTKPREEQYNSTYRVVSVLTVLHQDWLNGKEYKCKVSNKALPAPIEKTISKAKGQPREPQVCTLPPSRDELTKNQVSLSCAVKGFYPSDIAVEWESNGQPENNYKTTPPVLDSDGSFFLVSKLTVDKSRWQQGNVFSCSVMHEALHNHYTQKSLSLSPGK

SEQ ID NO: 57 - protein, 478 aa, Artificial Sequence
  57
DIVLTQSPDSLAVSLGERATINCKASQSVDYDGDSYMNWYQQKPGQPPKLLIYAASTLHSGIPDRFSGSGSGTDFTLTISSLQAEDVAVYYCQQSKEDPRTFGQGTKLEIKGGGGSGGGGSGGGGSEVQLVQSGAEVKKPGASVKVSCKASGYTFTDYNMDWVRQAPGKGLEWIGDINPNNGGTLYNQKFRGRVTLTVDKSISTAYMELSRLRSDDTAVYYCARSEVFYGNYADYWGQGTTVTVSSEPKSCDKTHTCPPCPAPEAAGGPSVFLFPPKPKDTLMISRTPEVTCVVVDVSHEDPEVKFNWYVDGVEVHNAKTKPREEQYNSTYRVVSVLTVLHQDWLNGKEYKCKVSNKALPAPIEKTISKAKGQPREPQVCTLPPSRDELTKNQVSLSCAVKGFYPSDIAVEWESNGQPENNYKTTPPVLDSDGSFFLVSKLTVDKSRWQQGNVFSCSVMHEALHNHYTQKSLSLSPGK

SEQ ID NO: 58 - protein, 478 aa, Artificial Sequence
  58
DIVLTQTPLSLSVTPGQPASISCKASQSVDYDGDSYMNWYLQKPGQPPQLLIYAASTLHSGVPDRFSGSGSGTDFTLKISRVEAEDVGVYYCQQSKEDPRTFGQGTKLEIKGGGGSGGGGSGGGGSEVQLVQSGAEVKKPGASVKVSCKASGYTFTDYNMDWVRQAPGQGLEWMGDINPNNGGTLYNQKFRGRVTMTVDTSISTAYMELSRLRSDDTAVYYCARSEVFYGNYADYWGQGTTVTVSSEPKSCDKTHTCPPCPAPEAAGGPSVFLFPPKPKDTLMISRTPEVTCVVVDVSHEDPEVKFNWYVDGVEVHNAKTKPREEQYNSTYRVVSVLTVLHQDWLNGKEYKCKVSNKALPAPIEKTISKAKGQPREPQVCTLPPSRDELTKNQVSLSCAVKGFYPSDIAVEWESNGQPENNYKTTPPVLDSDGSFFLVSKLTVDKSRWQQGNVFSCSVMHEALHNHYTQKSLSLSPGK

SEQ ID NO: 59 - protein, 478 aa, Artificial Sequence
  59
DIVLTQTPLSLSVTPGQPASISCKASQSVDYDGDSYMNWYLQKPGQPPQLLIYAASTLHSGVPDRFSGSGSGTDFTLKISRVEAEDVGVYYCQQSKEDPRTFGQGTKLEIKGGGGSGGGGSGGGGSEVQLVQSGAEVKKPGASVKVSCKASGYTFTDYNMDWVRQAPGQGLEWIGDINPNNGGTLYNQKFRGRVTLTVDTSISTAYMELSRLRSDDTAVYYCARSEVFYGNYADYWGQGTTVTVSSEPKSCDKTHTCPPCPAPEAAGGPSVFLFPPKPKDTLMISRTPEVTCVVVDVSHEDPEVKFNWYVDGVEVHNAKTKPREEQYNSTYRVVSVLTVLHQDWLNGKEYKCKVSNKALPAPIEKTISKAKGQPREPQVCTLPPSRDELTKNQVSLSCAVKGFYPSDIAVEWESNGQPENNYKTTPPVLDSDGSFFLVSKLTVDKSRWQQGNVFSCSVMHEALHNHYTQKSLSLSPGK

SEQ ID NO: 60 - protein, 478 aa, Artificial Sequence
  60
DIVLTQTPLSLSVTPGQPASISCKASQSVDYDGDSYMNWYLQKPGQPPQLLIYAASTLHSGVPDRFSGSGSGTDFTLKISRVEAEDVGVYYCQQSKEDPRTFGQGTKLEIKGGGGSGGGGSGGGGSEVQLVQSGAEVKKPGASVKVSCKASGYTFTDYNMDWVRQAPGQGLEWIGDINPNNGGTLYNQKFRGRVTLTVDKSISTAYMELSRLRSDDTAVYYCARSEVFYGNYADYWGQGTTVTVSSEPKSCDKTHTCPPCPAPEAAGGPSVFLFPPKPKDTLMISRTPEVTCVVVDVSHEDPEVKFNWYVDGVEVHNAKTKPREEQYNSTYRVVSVLTVLHQDWLNGKEYKCKVSNKALPAPIEKTISKAKGQPREPQVCTLPPSRDELTKNQVSLSCAVKGFYPSDIAVEWESNGQPENNYKTTPPVLDSDGSFFLVSKLTVDKSRWQQGNVFSCSVMHEALHNHYTQKSLSLSPGK

SEQ ID NO: 61 - protein, 478 aa, Artificial Sequence
  61
DIVLTQTPLSLSVTPGQPASISCKASQSVDYDGDSYMNWYLQKPGQPPQLLIYAASTLHSGVPDRFSGSGSGTDFTLKISRVEAEDVGVYYCQQSKEDPRTFGQGTKLEIKGGGGSGGGGSGGGGSEVQLVQSGAEVKKPGASVKVSCKASGYTFTDYNMDWVRQAPGKGLEWIGDINPNNGGTLYNQKFRGRVTLTVDKSISTAYMELSRLRSDDTAVYYCARSEVFYGNYADYWGQGTTVTVSSEPKSCDKTHTCPPCPAPEAAGGPSVFLFPPKPKDTLMISRTPEVTCVVVDVSHEDPEVKFNWYVDGVEVHNAKTKPREEQYNSTYRVVSVLTVLHQDWLNGKEYKCKVSNKALPAPIEKTISKAKGQPREPQVCTLPPSRDELTKNQVSLSCAVKGFYPSDIAVEWESNGQPENNYKTTPPVLDSDGSFFLVSKLTVDKSRWQQGNVFSCSVMHEALHNHYTQKSLSLSPGK

SEQ ID NO: 62 - protein, 478 aa, Artificial Sequence
  62
DIVLTQTPLSLSVTPGQPASISCKASQSVDYDGDSYMNWYLQKPGQPPQLLIYAASTLHSGIPDRFSGSGSGTDFTLKISRVEAEDVGVYYCQQSKEDPRTFGQGTKLEIKGGGGSGGGGSGGGGSEVQLVQSGAEVKKPGASVKVSCKASGYTFTDYNMDWVRQAPGQGLEWMGDINPNNGGTLYNQKFRGRVTMTVDTSISTAYMELSRLRSDDTAVYYCARSEVFYGNYADYWGQGTTVTVSSEPKSCDKTHTCPPCPAPEAAGGPSVFLFPPKPKDTLMISRTPEVTCVVVDVSHEDPEVKFNWYVDGVEVHNAKTKPREEQYNSTYRVVSVLTVLHQDWLNGKEYKCKVSNKALPAPIEKTISKAKGQPREPQVCTLPPSRDELTKNQVSLSCAVKGFYPSDIAVEWESNGQPENNYKTTPPVLDSDGSFFLVSKLTVDKSRWQQGNVFSCSVMHEALHNHYTQKSLSLSPGK

SEQ ID NO: 63 - protein, 478 aa, Artificial Sequence
  63
DIVLTQTPLSLSVTPGQPASISCKASQSVDYDGDSYMNWYLQKPGQPPQLLIYAASTLHSGIPDRFSGSGSGTDFTLKISRVEAEDVGVYYCQQSKEDPRTFGQGTKLEIKGGGGSGGGGSGGGGSEVQLVQSGAEVKKPGASVKVSCKASGYTFTDYNMDWVRQAPGQGLEWIGDINPNNGGTLYNQKFRGRVTLTVDTSISTAYMELSRLRSDDTAVYYCARSEVFYGNYADYWGQGTTVTVSSEPKSCDKTHTCPPCPAPEAAGGPSVFLFPPKPKDTLMISRTPEVTCVVVDVSHEDPEVKFNWYVDGVEVHNAKTKPREEQYNSTYRVVSVLTVLHQDWLNGKEYKCKVSNKALPAPIEKTISKAKGQPREPQVCTLPPSRDELTKNQVSLSCAVKGFYPSDIAVEWESNGQPENNYKTTPPVLDSDGSFFLVSKLTVDKSRWQQGNVFSCSVMHEALHNHYTQKSLSLSPGK

SEQ ID NO: 64 - protein, 478 aa, Artificial Sequence
  64
DIVLTQTPLSLSVTPGQPASISCKASQSVDYDGDSYMNWYLQKPGQPPQLLIYAASTLHSGIPDRFSGSGSGTDFTLKISRVEAEDVGVYYCQQSKEDPRTFGQGTKLEIKGGGGSGGGGSGGGGSEVQLVQSGAEVKKPGASVKVSCKASGYTFTDYNMDWVRQAPGQGLEWIGDINPNNGGTLYNQKFRGRVTLTVDKSISTAYMELSRLRSDDTAVYYCARSEVFYGNYADYWGQGTTVTVSSEPKSCDKTHTCPPCPAPEAAGGPSVFLFPPKPKDTLMISRTPEVTCVVVDVSHEDPEVKFNWYVDGVEVHNAKTKPREEQYNSTYRVVSVLTVLHQDWLNGKEYKCKVSNKALPAPIEKTISKAKGQPREPQVCTLPPSRDELTKNQVSLSCAVKGFYPSDIAVEWESNGQPENNYKTTPPVLDSDGSFFLVSKLTVDKSRWQQGNVFSCSVMHEALHNHYTQKSLSLSPGK

SEQ ID NO: 65 - protein, 478 aa, Artificial Sequence
  65
DIVLTQTPLSLSVTPGQPASISCKASQSVDYDGDSYMNWYLQKPGQPPQLLIYAASTLHSGIPDRFSGSGSGTDFTLKISRVEAEDVGVYYCQQSKEDPRTFGQGTKLEIKGGGGSGGGGSGGGGSEVQLVQSGAEVKKPGASVKVSCKASGYTFTDYNMDWVRQAPGKGLEWIGDINPNNGGTLYNQKFRGRVTLTVDKSISTAYMELSRLRSDDTAVYYCARSEVFYGNYADYWGQGTTVTVSSEPKSCDKTHTCPPCPAPEAAGGPSVFLFPPKPKDTLMISRTPEVTCVVVDVSHEDPEVKFNWYVDGVEVHNAKTKPREEQYNSTYRVVSVLTVLHQDWLNGKEYKCKVSNKALPAPIEKTISKAKGQPREPQVCTLPPSRDELTKNQVSLSCAVKGFYPSDIAVEWESNGQPENNYKTTPPVLDSDGSFFLVSKLTVDKSRWQQGNVFSCSVMHEALHNHYTQKSLSLSPGK

SEQ ID NO: 66 - protein, 478 aa, Artificial Sequence
  66
DIVLTQSPVSLAVPLGQRATISCKASQSVDYDGDSYMNWYQQKPGQPPKLLIYAASTLHSGIPVRFSGSGSGTDFTLNIHPVEEEDAASYYCQQSKEDPRTFGGGTKLEIKGGGGSGGGGSGGGGSEVLLQQSGPEVVKPGASVKITCKASGYTFTDYNMDWVKQSHGKSLEWIGDINPNNAGTLYNQKFRGRVTLIVDKSSSTAYMELRSLTSDDTAVYYCARSEVFYGNYADYWGQGTTLTVSSEPKSCDKTHTCPPCPAPEAAGGPSVFLFPPKPKDTLMISRTPEVTCVVVDVSHEDPEVKFNWYVDGVEVHNAKTKPREEQYNSTYRVVSVLTVLHQDWLNGKEYKCKVSNKALPAPIEKTISKAKGQPREPQVCTLPPSRDELTKNQVSLSCAVKGFYPSDIAVEWESNGQPENNYKTTPPVLDSDGSFFLVSKLTVDKSRWQQGNVFSCSVMHEALHNHYTQKSLSLSPGK

SEQ ID NO: 67 - protein, 478 aa, Artificial Sequence
  67
DIVLTQSPVSLAVPLGQRATISCKASQSVDYDADSYMNWYQQKPGQPPKLLIYAASTLHSGIPVRFSGSGSGTDFTLNIHPVEEEDAASYYCQQSKEDPRTFGGGTKLEIKGGGGSGGGGSGGGGSEVLLQQSGPEVVKPGASVKITCKASGYTFTDYNMDWVKQSHGKSLEWIGDINPNNGGTLYNQKFRGRVTLIVDKSSSTAYMELRSLTSDDTAVYYCARSEVFYGNYADYWGQGTTLTVSSEPKSCDKTHTCPPCPAPEAAGGPSVFLFPPKPKDTLMISRTPEVTCVVVDVSHEDPEVKFNWYVDGVEVHNAKTKPREEQYNSTYRVVSVLTVLHQDWLNGKEYKCKVSNKALPAPIEKTISKAKGQPREPQVCTLPPSRDELTKNQVSLSCAVKGFYPSDIAVEWESNGQPENNYKTTPPVLDSDGSFFLVSKLTVDKSRWQQGNVFSCSVMHEALHNHYTQKSLSLSPGK

SEQ ID NO: 68 - protein, 20 aa, Artificial Sequence
  68
METDTLLLWVLLLWVPGSTG

SEQ ID NO: 69 - DNA, 1449 bp, Artificial Sequence
  69
caggccgtggtgacccaggagccctccctgaccgtgtcccccggcggcaccgtgaccctgacctgcaggtcctccaccggcgccgtgaccacctccaactacgccaactgggtgcagcagaagcccggccaggcccccaggggcctgatcggcggcaccaacaagagggccccctggacccccgccaggttctccggctccctgctgggcggcaaggccgccctgaccatcaccggcgcccaggccgaggacgaggccgactactactgcgccctgtggtactccaacctgtgggtgttcggcggcggcaccaagctgaccgtgctgggcggaggcggtggatcaggcggaggtggctcaggtggaggcggttctgaggtgcagctggtggagtccggcggcggcctggtgcagcccggcggctccctgaggctgtcctgcgccgcctccggcttcaccttcaacacctacgccatgaactgggtgaggcaggcccccggcaagggcctggagtgggtggccaggatcaggtccaagtacaacaactacgccacctactacgccgactccgtgaaggacaggttcaccatctccagggacgactccaagaactccctgtacctgcagatgaactccctgaagaccgaggacaccgccgtgtactactgcgtgaggcacggcaacttcggcaactcctacgtgtcctggttcgcctactggggccagggcaccctggtgaccgtgtcctccgagcccaagtcctgcgacaagacccacacctgccccccctgccccgcccccgaggccgccggcggcccctccgtgttcctgttcccccccaagcccaaggacaccctgatgatctccaggacccccgaggtgacctgcgtggtggtggacgtgtcccacgaggaccccgaggtgaagttcaactggtacgtggacggcgtggaggtgcacaacgccaagaccaagcccagggaggagcagtacaactccacctacagggtggtgtccgtgctgaccgtgctgcaccaggactggctgaacggcaaggagtacaagtgcaaggtgtccaacaaggccctgcccgcccccatcgagaagaccatctccaaggccaagggccagcccagggagccccaggtgtacaccctgcccccctgcagggacgagctgaccaagaaccaggtgtccctgtggtgcctggtgaagggcttctacccctccgacatcgccgtggagtgggagtccaacggccagcccgagaacaactacaagaccaccccccccgtgctggactccgacggctccttcttcctgtactccaagctgaccgtggacaagtccaggtggcagcagggcaacgtgttctcctgctccgtgatgcacgaggccctgcacaaccactacacccagaagtccctgtccctgtcccccggcaagtaa

SEQ ID NO: 70 - DNA, 1437 bp, Artificial Sequence
  70
gacatcgtgctgacccagtcccccgactccctggccgtgtccctgggcgagagggccaccatcaactgcaaggcctcccagtccgtggactacgacggcgactcctacatgaactggtaccagcagaagcccggccagccccccaagctgctgatctacgccgcctccaccctgcactccggcgtgcccgacaggttctccggctccggctccggcaccgacttcaccctgaccatctcctccctgcaggccgaggacgtggccgtgtactactgccagcagtccaaggaggaccccaggaccttcggccagggcaccaagctggagatcaagggaggcggtggatcaggcggaggtggctcaggtggaggcggttctgaggtgcagctggtgcagtccggcgccgaggtgaagaagcccggcgcctccgtgaaggtgtcctgcaaggcctccggctacaccttcaccgactacaacatggactgggtgaggcaggcccccggccagggcctggagtggatgggcgacatcaaccccaacaacggcggcaccctgtacaaccagaagttcaggggcagggtgaccatgaccgtggacacctccatctccaccgcctacatggagctgtccaggctgaggtccgacgacaccgccgtgtactactgcgccaggtccgaggtgttctacggcaactacgccgactactggggccagggcaccaccgtgaccgtgtcctccgagcccaagtcctgcgacaagacccacacctgccccccctgccccgcccccgaggccgccggcggcccctccgtgttcctgttcccccccaagcccaaggacaccctgatgatctccaggacccccgaggtgacctgcgtggtggtggacgtgtcccacgaggaccccgaggtgaagttcaactggtacgtggacggcgtggaggtgcacaacgccaagaccaagcccagggaggagcagtacaactccacctacagggtggtgtccgtgctgaccgtgctgcaccaggactggctgaacggcaaggagtacaagtgcaaggtgtccaacaaggccctgcccgcccccatcgagaagaccatctccaaggccaagggccagcccagggagccccaggtgtgcaccctgcccccctccagggacgagctgaccaagaaccaggtgtccctgtcctgcgccgtgaagggcttctacccctccgacatcgccgtggagtgggagtccaacggccagcccgagaacaactacaagaccaccccccccgtgctggactccgacggctccttcttcctggtgtccaagctgaccgtggacaagtccaggtggcagcagggcaacgtgttctcctgctccgtgatgcacgaggccctgcacaaccactacacccagaagtccctgtccctgtcccccggcaagtaa

SEQ ID NO: 71 - DNA, 1437 bp, Artificial Sequence
  71
gacatcgtgctgacccagtcccccgactccctggccgtgtccctgggcgagagggccaccatcaactgcaaggcctcccagtccgtggactacgacggcgactcctacatgaactggtaccagcagaagcccggccagccccccaagctgctgatctacgccgcctccaccctgcactccggcgtgcccgacaggttctccggctccggctccggcaccgacttcaccctgaccatctcctccctgcaggccgaggacgtggccgtgtactactgccagcagtccaaggaggaccccaggaccttcggccagggcaccaagctggagatcaagggaggcggtggatcaggcggaggtggctcaggtggaggcggttctgaggtgcagctggtgcagtccggcgccgaggtgaagaagcccggcgcctccgtgaaggtgtcctgcaaggcctccggctacaccttcaccgactacaacatggactgggtgaggcaggcccccggccagggcctggagtggatcggcgacatcaaccccaacaacggcggcaccctgtacaaccagaagttcaggggcagggtgaccctgaccgtggacacctccatctccaccgcctacatggagctgtccaggctgaggtccgacgacaccgccgtgtactactgcgccaggtccgaggtgttctacggcaactacgccgactactggggccagggcaccaccgtgaccgtgtcctccgagcccaagtcctgcgacaagacccacacctgccccccctgccccgcccccgaggccgccggcggcccctccgtgttcctgttcccccccaagcccaaggacaccctgatgatctccaggacccccgaggtgacctgcgtggtggtggacgtgtcccacgaggaccccgaggtgaagttcaactggtacgtggacggcgtggaggtgcacaacgccaagaccaagcccagggaggagcagtacaactccacctacagggtggtgtccgtgctgaccgtgctgcaccaggactggctgaacggcaaggagtacaagtgcaaggtgtccaacaaggccctgcccgcccccatcgagaagaccatctccaaggccaagggccagcccagggagccccaggtgtgcaccctgcccccctccagggacgagctgaccaagaaccaggtgtccctgtcctgcgccgtgaagggcttctacccctccgacatcgccgtggagtgggagtccaacggccagcccgagaacaactacaagaccaccccccccgtgctggactccgacggctccttcttcctggtgtccaagctgaccgtggacaagtccaggtggcagcagggcaacgtgttctcctgctccgtgatgcacgaggccctgcacaaccactacacccagaagtccctgtccctgtcccccggcaagtaa

SEQ ID NO: 72 - DNA, 1437 bp, Artificial Sequence
  72
gacatcgtgctgacccagtcccccgactccctggccgtgtccctgggcgagagggccaccatcaactgcaaggcctcccagtccgtggactacgacggcgactcctacatgaactggtaccagcagaagcccggccagccccccaagctgctgatctacgccgcctccaccctgcactccggcgtgcccgacaggttctccggctccggctccggcaccgacttcaccctgaccatctcctccctgcaggccgaggacgtggccgtgtactactgccagcagtccaaggaggaccccaggaccttcggccagggcaccaagctggagatcaagggaggcggtggatcaggcggaggtggctcaggtggaggcggttctgaggtgcagctggtgcagtccggcgccgaggtgaagaagcccggcgcctccgtgaaggtgtcctgcaaggcctccggctacaccttcaccgactacaacatggactgggtgaggcaggcccccggccagggcctggagtggatcggcgacatcaaccccaacaacggcggcaccctgtacaaccagaagttcaggggcagggtgaccctgaccgtggacaagtccatctccaccgcctacatggagctgtccaggctgaggtccgacgacaccgccgtgtactactgcgccaggtccgaggtgttctacggcaactacgccgactactggggccagggcaccaccgtgaccgtgtcctccgagcccaagtcctgcgacaagacccacacctgccccccctgccccgcccccgaggccgccggcggcccctccgtgttcctgttcccccccaagcccaaggacaccctgatgatctccaggacccccgaggtgacctgcgtggtggtggacgtgtcccacgaggaccccgaggtgaagttcaactggtacgtggacggcgtggaggtgcacaacgccaagaccaagcccagggaggagcagtacaactccacctacagggtggtgtccgtgctgaccgtgctgcaccaggactggctgaacggcaaggagtacaagtgcaaggtgtccaacaaggccctgcccgcccccatcgagaagaccatctccaaggccaagggccagcccagggagccccaggtgtgcaccctgcccccctccagggacgagctgaccaagaaccaggtgtccctgtcctgcgccgtgaagggcttctacccctccgacatcgccgtggagtgggagtccaacggccagcccgagaacaactacaagaccaccccccccgtgctggactccgacggctccttcttcctggtgtccaagctgaccgtggacaagtccaggtggcagcagggcaacgtgttctcctgctccgtgatgcacgaggccctgcacaaccactacacccagaagtccctgtccctgtcccccggcaagtaa

SEQ ID NO: 73 - DNA, 1437 bp, Artificial Sequence
  73
gacatcgtgctgacccagtcccccgactccctggccgtgtccctgggcgagagggccaccatcaactgcaaggcctcccagtccgtggactacgacggcgactcctacatgaactggtaccagcagaagcccggccagccccccaagctgctgatctacgccgcctccaccctgcactccggcgtgcccgacaggttctccggctccggctccggcaccgacttcaccctgaccatctcctccctgcaggccgaggacgtggccgtgtactactgccagcagtccaaggaggaccccaggaccttcggccagggcaccaagctggagatcaagggaggcggtggatcaggcggaggtggctcaggtggaggcggttctgaggtgcagctggtgcagtccggcgccgaggtgaagaagcccggcgcctccgtgaaggtgtcctgcaaggcctccggctacaccttcaccgactacaacatggactgggtgaggcaggcccccggcaagggcctggagtggatcggcgacatcaaccccaacaacggcggcaccctgtacaaccagaagttcaggggcagggtgaccctgaccgtggacaagtccatctccaccgcctacatggagctgtccaggctgaggtccgacgacaccgccgtgtactactgcgccaggtccgaggtgttctacggcaactacgccgactactggggccagggcaccaccgtgaccgtgtcctccgagcccaagtcctgcgacaagacccacacctgccccccctgccccgcccccgaggccgccggcggcccctccgtgttcctgttcccccccaagcccaaggacaccctgatgatctccaggacccccgaggtgacctgcgtggtggtggacgtgtcccacgaggaccccgaggtgaagttcaactggtacgtggacggcgtggaggtgcacaacgccaagaccaagcccagggaggagcagtacaactccacctacagggtggtgtccgtgctgaccgtgctgcaccaggactggctgaacggcaaggagtacaagtgcaaggtgtccaacaaggccctgcccgcccccatcgagaagaccatctccaaggccaagggccagcccagggagccccaggtgtgcaccctgcccccctccagggacgagctgaccaagaaccaggtgtccctgtcctgcgccgtgaagggcttctacccctccgacatcgccgtggagtgggagtccaacggccagcccgagaacaactacaagaccaccccccccgtgctggactccgacggctccttcttcctggtgtccaagctgaccgtggacaagtccaggtggcagcagggcaacgtgttctcctgctccgtgatgcacgaggccctgcacaaccactacacccagaagtccctgtccctgtcccccggcaagtaa

SEQ ID NO: 74 - DNA, 1437 bp, Artificial Sequence
  74
gacatcgtgctgacccagtcccccgactccctggccgtgtccctgggcgagagggccaccatcaactgcaaggcctcccagtccgtggactacgacggcgactcctacatgaactggtaccagcagaagcccggccagccccccaagctgctgatctacgccgcctccaccctgcactccggcatccccgacaggttctccggctccggctccggcaccgacttcaccctgaccatctcctccctgcaggccgaggacgtggccgtgtactactgccagcagtccaaggaggaccccaggaccttcggccagggcaccaagctggagatcaagggaggcggtggatcaggcggaggtggctcaggtggaggcggttctgaggtgcagctggtgcagtccggcgccgaggtgaagaagcccggcgcctccgtgaaggtgtcctgcaaggcctccggctacaccttcaccgactacaacatggactgggtgaggcaggcccccggccagggcctggagtggatgggcgacatcaaccccaacaacggcggcaccctgtacaaccagaagttcaggggcagggtgaccatgaccgtggacacctccatctccaccgcctacatggagctgtccaggctgaggtccgacgacaccgccgtgtactactgcgccaggtccgaggtgttctacggcaactacgccgactactggggccagggcaccaccgtgaccgtgtcctccgagcccaagtcctgcgacaagacccacacctgccccccctgccccgcccccgaggccgccggcggcccctccgtgttcctgttcccccccaagcccaaggacaccctgatgatctccaggacccccgaggtgacctgcgtggtggtggacgtgtcccacgaggaccccgaggtgaagttcaactggtacgtggacggcgtggaggtgcacaacgccaagaccaagcccagggaggagcagtacaactccacctacagggtggtgtccgtgctgaccgtgctgcaccaggactggctgaacggcaaggagtacaagtgcaaggtgtccaacaaggccctgcccgcccccatcgagaagaccatctccaaggccaagggccagcccagggagccccaggtgtgcaccctgcccccctccagggacgagctgaccaagaaccaggtgtccctgtcctgcgccgtgaagggcttctacccctccgacatcgccgtggagtgggagtccaacggccagcccgagaacaactacaagaccaccccccccgtgctggactccgacggctccttcttcctggtgtccaagctgaccgtggacaagtccaggtggcagcagggcaacgtgttctcctgctccgtgatgcacgaggccctgcacaaccactacacccagaagtccctgtccctgtcccccggcaagtaa

SEQ ID NO: 75 - DNA, 1437 bp, Artificial Sequence
  75
gacatcgtgctgacccagtcccccgactccctggccgtgtccctgggcgagagggccaccatcaactgcaaggcctcccagtccgtggactacgacggcgactcctacatgaactggtaccagcagaagcccggccagccccccaagctgctgatctacgccgcctccaccctgcactccggcatccccgacaggttctccggctccggctccggcaccgacttcaccctgaccatctcctccctgcaggccgaggacgtggccgtgtactactgccagcagtccaaggaggaccccaggaccttcggccagggcaccaagctggagatcaagggaggcggtggatcaggcggaggtggctcaggtggaggcggttctgaggtgcagctggtgcagtccggcgccgaggtgaagaagcccggcgcctccgtgaaggtgtcctgcaaggcctccggctacaccttcaccgactacaacatggactgggtgaggcaggcccccggccagggcctggagtggatcggcgacatcaaccccaacaacggcggcaccctgtacaaccagaagttcaggggcagggtgaccctgaccgtggacacctccatctccaccgcctacatggagctgtccaggctgaggtccgacgacaccgccgtgtactactgcgccaggtccgaggtgttctacggcaactacgccgactactggggccagggcaccaccgtgaccgtgtcctccgagcccaagtcctgcgacaagacccacacctgccccccctgccccgcccccgaggccgccggcggcccctccgtgttcctgttcccccccaagcccaaggacaccctgatgatctccaggacccccgaggtgacctgcgtggtggtggacgtgtcccacgaggaccccgaggtgaagttcaactggtacgtggacggcgtggaggtgcacaacgccaagaccaagcccagggaggagcagtacaactccacctacagggtggtgtccgtgctgaccgtgctgcaccaggactggctgaacggcaaggagtacaagtgcaaggtgtccaacaaggccctgcccgcccccatcgagaagaccatctccaaggccaagggccagcccagggagccccaggtgtgcaccctgcccccctccagggacgagctgaccaagaaccaggtgtccctgtcctgcgccgtgaagggcttctacccctccgacatcgccgtggagtgggagtccaacggccagcccgagaacaactacaagaccaccccccccgtgctggactccgacggctccttcttcctggtgtccaagctgaccgtggacaagtccaggtggcagcagggcaacgtgttctcctgctccgtgatgcacgaggccctgcacaaccactacacccagaagtccctgtccctgtcccccggcaagtaa

SEQ ID NO: 76 - DNA, 1437 bp, Artificial Sequence
  76
gacatcgtgctgacccagtcccccgactccctggccgtgtccctgggcgagagggccaccatcaactgcaaggcctcccagtccgtggactacgacggcgactcctacatgaactggtaccagcagaagcccggccagccccccaagctgctgatctacgccgcctccaccctgcactccggcatccccgacaggttctccggctccggctccggcaccgacttcaccctgaccatctcctccctgcaggccgaggacgtggccgtgtactactgccagcagtccaaggaggaccccaggaccttcggccagggcaccaagctggagatcaagggaggcggtggatcaggcggaggtggctcaggtggaggcggttctgaggtgcagctggtgcagtccggcgccgaggtgaagaagcccggcgcctccgtgaaggtgtcctgcaaggcctccggctacaccttcaccgactacaacatggactgggtgaggcaggcccccggccagggcctggagtggatcggcgacatcaaccccaacaacggcggcaccctgtacaaccagaagttcaggggcagggtgaccctgaccgtggacaagtccatctccaccgcctacatggagctgtccaggctgaggtccgacgacaccgccgtgtactactgcgccaggtccgaggtgttctacggcaactacgccgactactggggccagggcaccaccgtgaccgtgtcctccgagcccaagtcctgcgacaagacccacacctgccccccctgccccgcccccgaggccgccggcggcccctccgtgttcctgttcccccccaagcccaaggacaccctgatgatctccaggacccccgaggtgacctgcgtggtggtggacgtgtcccacgaggaccccgaggtgaagttcaactggtacgtggacggcgtggaggtgcacaacgccaagaccaagcccagggaggagcagtacaactccacctacagggtggtgtccgtgctgaccgtgctgcaccaggactggctgaacggcaaggagtacaagtgcaaggtgtccaacaaggccctgcccgcccccatcgagaagaccatctccaaggccaagggccagcccagggagccccaggtgtgcaccctgcccccctccagggacgagctgaccaagaaccaggtgtccctgtcctgcgccgtgaagggcttctacccctccgacatcgccgtggagtgggagtccaacggccagcccgagaacaactacaagaccaccccccccgtgctggactccgacggctccttcttcctggtgtccaagctgaccgtggacaagtccaggtggcagcagggcaacgtgttctcctgctccgtgatgcacgaggccctgcacaaccactacacccagaagtccctgtccctgtcccccggcaagtaa

SEQ ID NO: 77 - DNA, 1437 bp, Artificial Sequence
  77
gacatcgtgctgacccagtcccccgactccctggccgtgtccctgggcgagagggccaccatcaactgcaaggcctcccagtccgtggactacgacggcgactcctacatgaactggtaccagcagaagcccggccagccccccaagctgctgatctacgccgcctccaccctgcactccggcatccccgacaggttctccggctccggctccggcaccgacttcaccctgaccatctcctccctgcaggccgaggacgtggccgtgtactactgccagcagtccaaggaggaccccaggaccttcggccagggcaccaagctggagatcaagggaggcggtggatcaggcggaggtggctcaggtggaggcggttctgaggtgcagctggtgcagtccggcgccgaggtgaagaagcccggcgcctccgtgaaggtgtcctgcaaggcctccggctacaccttcaccgactacaacatggactgggtgaggcaggcccccggcaagggcctggagtggatcggcgacatcaaccccaacaacggcggcaccctgtacaaccagaagttcaggggcagggtgaccctgaccgtggacaagtccatctccaccgcctacatggagctgtccaggctgaggtccgacgacaccgccgtgtactactgcgccaggtccgaggtgttctacggcaactacgccgactactggggccagggcaccaccgtgaccgtgtcctccgagcccaagtcctgcgacaagacccacacctgccccccctgccccgcccccgaggccgccggcggcccctccgtgttcctgttcccccccaagcccaaggacaccctgatgatctccaggacccccgaggtgacctgcgtggtggtggacgtgtcccacgaggaccccgaggtgaagttcaactggtacgtggacggcgtggaggtgcacaacgccaagaccaagcccagggaggagcagtacaactccacctacagggtggtgtccgtgctgaccgtgctgcaccaggactggctgaacggcaaggagtacaagtgcaaggtgtccaacaaggccctgcccgcccccatcgagaagaccatctccaaggccaagggccagcccagggagccccaggtgtgcaccctgcccccctccagggacgagctgaccaagaaccaggtgtccctgtcctgcgccgtgaagggcttctacccctccgacatcgccgtggagtgggagtccaacggccagcccgagaacaactacaagaccaccccccccgtgctggactccgacggctccttcttcctggtgtccaagctgaccgtggacaagtccaggtggcagcagggcaacgtgttctcctgctccgtgatgcacgaggccctgcacaaccactacacccagaagtccctgtccctgtcccccggcaagtaa

SEQ ID NO: 78 - DNA, 1437 bp, Artificial Sequence
  78
gacatcgtgctgacccagacccccctgtccctgtccgtgacccccggccagcccgcctccatctcctgcaaggcctcccagtccgtggactacgacggcgactcctacatgaactggtacctgcagaagcccggccagcccccccagctgctgatctacgccgcctccaccctgcactccggcgtgcccgacaggttctccggctccggctccggcaccgacttcaccctgaagatctccagggtggaggccgaggacgtgggcgtgtactactgccagcagtccaaggaggaccccaggaccttcggccagggcaccaagctggagatcaagggaggcggtggatcaggcggaggtggctcaggtggaggcggttctgaggtgcagctggtgcagtccggcgccgaggtgaagaagcccggcgcctccgtgaaggtgtcctgcaaggcctccggctacaccttcaccgactacaacatggactgggtgaggcaggcccccggccagggcctggagtggatgggcgacatcaaccccaacaacggcggcaccctgtacaaccagaagttcaggggcagggtgaccatgaccgtggacacctccatctccaccgcctacatggagctgtccaggctgaggtccgacgacaccgccgtgtactactgcgccaggtccgaggtgttctacggcaactacgccgactactggggccagggcaccaccgtgaccgtgtcctccgagcccaagtcctgcgacaagacccacacctgccccccctgccccgcccccgaggccgccggcggcccctccgtgttcctgttcccccccaagcccaaggacaccctgatgatctccaggacccccgaggtgacctgcgtggtggtggacgtgtcccacgaggaccccgaggtgaagttcaactggtacgtggacggcgtggaggtgcacaacgccaagaccaagcccagggaggagcagtacaactccacctacagggtggtgtccgtgctgaccgtgctgcaccaggactggctgaacggcaaggagtacaagtgcaaggtgtccaacaaggccctgcccgcccccatcgagaagaccatctccaaggccaagggccagcccagggagccccaggtgtgcaccctgcccccctccagggacgagctgaccaagaaccaggtgtccctgtcctgcgccgtgaagggcttctacccctccgacatcgccgtggagtgggagtccaacggccagcccgagaacaactacaagaccaccccccccgtgctggactccgacggctccttcttcctggtgtccaagctgaccgtggacaagtccaggtggcagcagggcaacgtgttctcctgctccgtgatgcacgaggccctgcacaaccactacacccagaagtccctgtccctgtcccccggcaagtaa

SEQ ID NO: 79 - DNA, 1437 bp, Artificial Sequence
  79
gacatcgtgctgacccagacccccctgtccctgtccgtgacccccggccagcccgcctccatctcctgcaaggcctcccagtccgtggactacgacggcgactcctacatgaactggtacctgcagaagcccggccagcccccccagctgctgatctacgccgcctccaccctgcactccggcgtgcccgacaggttctccggctccggctccggcaccgacttcaccctgaagatctccagggtggaggccgaggacgtgggcgtgtactactgccagcagtccaaggaggaccccaggaccttcggccagggcaccaagctggagatcaagggaggcggtggatcaggcggaggtggctcaggtggaggcggttctgaggtgcagctggtgcagtccggcgccgaggtgaagaagcccggcgcctccgtgaaggtgtcctgcaaggcctccggctacaccttcaccgactacaacatggactgggtgaggcaggcccccggccagggcctggagtggatcggcgacatcaaccccaacaacggcggcaccctgtacaaccagaagttcaggggcagggtgaccctgaccgtggacacctccatctccaccgcctacatggagctgtccaggctgaggtccgacgacaccgccgtgtactactgcgccaggtccgaggtgttctacggcaactacgccgactactggggccagggcaccaccgtgaccgtgtcctccgagcccaagtcctgcgacaagacccacacctgccccccctgccccgcccccgaggccgccggcggcccctccgtgttcctgttcccccccaagcccaaggacaccctgatgatctccaggacccccgaggtgacctgcgtggtggtggacgtgtcccacgaggaccccgaggtgaagttcaactggtacgtggacggcgtggaggtgcacaacgccaagaccaagcccagggaggagcagtacaactccacctacagggtggtgtccgtgctgaccgtgctgcaccaggactggctgaacggcaaggagtacaagtgcaaggtgtccaacaaggccctgcccgcccccatcgagaagaccatctccaaggccaagggccagcccagggagccccaggtgtgcaccctgcccccctccagggacgagctgaccaagaaccaggtgtccctgtcctgcgccgtgaagggcttctacccctccgacatcgccgtggagtgggagtccaacggccagcccgagaacaactacaagaccaccccccccgtgctggactccgacggctccttcttcctggtgtccaagctgaccgtggacaagtccaggtggcagcagggcaacgtgttctcctgctccgtgatgcacgaggccctgcacaaccactacacccagaagtccctgtccctgtcccccggcaagtaa

SEQ ID NO: 80 - DNA, 1437 bp, Artificial Sequence
  80
gacatcgtgctgacccagacccccctgtccctgtccgtgacccccggccagcccgcctccatctcctgcaaggcctcccagtccgtggactacgacggcgactcctacatgaactggtacctgcagaagcccggccagcccccccagctgctgatctacgccgcctccaccctgcactccggcgtgcccgacaggttctccggctccggctccggcaccgacttcaccctgaagatctccagggtggaggccgaggacgtgggcgtgtactactgccagcagtccaaggaggaccccaggaccttcggccagggcaccaagctggagatcaagggaggcggtggatcaggcggaggtggctcaggtggaggcggttctgaggtgcagctggtgcagtccggcgccgaggtgaagaagcccggcgcctccgtgaaggtgtcctgcaaggcctccggctacaccttcaccgactacaacatggactgggtgaggcaggcccccggccagggcctggagtggatcggcgacatcaaccccaacaacggcggcaccctgtacaaccagaagttcaggggcagggtgaccctgaccgtggacaagtccatctccaccgcctacatggagctgtccaggctgaggtccgacgacaccgccgtgtactactgcgccaggtccgaggtgttctacggcaactacgccgactactggggccagggcaccaccgtgaccgtgtcctccgagcccaagtcctgcgacaagacccacacctgccccccctgccccgcccccgaggccgccggcggcccctccgtgttcctgttcccccccaagcccaaggacaccctgatgatctccaggacccccgaggtgacctgcgtggtggtggacgtgtcccacgaggaccccgaggtgaagttcaactggtacgtggacggcgtggaggtgcacaacgccaagaccaagcccagggaggagcagtacaactccacctacagggtggtgtccgtgctgaccgtgctgcaccaggactggctgaacggcaaggagtacaagtgcaaggtgtccaacaaggccctgcccgcccccatcgagaagaccatctccaaggccaagggccagcccagggagccccaggtgtgcaccctgcccccctccagggacgagctgaccaagaaccaggtgtccctgtcctgcgccgtgaagggcttctacccctccgacatcgccgtggagtgggagtccaacggccagcccgagaacaactacaagaccaccccccccgtgctggactccgacggctccttcttcctggtgtccaagctgaccgtggacaagtccaggtggcagcagggcaacgtgttctcctgctccgtgatgcacgaggccctgcacaaccactacacccagaagtccctgtccctgtcccccggcaagtaa

SEQ ID NO: 81 - DNA, 1437 bp, Artificial Sequence
  81
gacatcgtgctgacccagacccccctgtccctgtccgtgacccccggccagcccgcctccatctcctgcaaggcctcccagtccgtggactacgacggcgactcctacatgaactggtacctgcagaagcccggccagcccccccagctgctgatctacgccgcctccaccctgcactccggcgtgcccgacaggttctccggctccggctccggcaccgacttcaccctgaagatctccagggtggaggccgaggacgtgggcgtgtactactgccagcagtccaaggaggaccccaggaccttcggccagggcaccaagctggagatcaagggaggcggtggatcaggcggaggtggctcaggtggaggcggttctgaggtgcagctggtgcagtccggcgccgaggtgaagaagcccggcgcctccgtgaaggtgtcctgcaaggcctccggctacaccttcaccgactacaacatggactgggtgaggcaggcccccggcaagggcctggagtggatcggcgacatcaaccccaacaacggcggcaccctgtacaaccagaagttcaggggcagggtgaccctgaccgtggacaagtccatctccaccgcctacatggagctgtccaggctgaggtccgacgacaccgccgtgtactactgcgccaggtccgaggtgttctacggcaactacgccgactactggggccagggcaccaccgtgaccgtgtcctccgagcccaagtcctgcgacaagacccacacctgccccccctgccccgcccccgaggccgccggcggcccctccgtgttcctgttcccccccaagcccaaggacaccctgatgatctccaggacccccgaggtgacctgcgtggtggtggacgtgtcccacgaggaccccgaggtgaagttcaactggtacgtggacggcgtggaggtgcacaacgccaagaccaagcccagggaggagcagtacaactccacctacagggtggtgtccgtgctgaccgtgctgcaccaggactggctgaacggcaaggagtacaagtgcaaggtgtccaacaaggccctgcccgcccccatcgagaagaccatctccaaggccaagggccagcccagggagccccaggtgtgcaccctgcccccctccagggacgagctgaccaagaaccaggtgtccctgtcctgcgccgtgaagggcttctacccctccgacatcgccgtggagtgggagtccaacggccagcccgagaacaactacaagaccaccccccccgtgctggactccgacggctccttcttcctggtgtccaagctgaccgtggacaagtccaggtggcagcagggcaacgtgttctcctgctccgtgatgcacgaggccctgcacaaccactacacccagaagtccctgtccctgtcccccggcaagtaa

SEQ ID NO: 82 - DNA, 1437 bp, Artificial Sequence
  82
gacatcgtgctgacccagacccccctgtccctgtccgtgacccccggccagcccgcctccatctcctgcaaggcctcccagtccgtggactacgacggcgactcctacatgaactggtacctgcagaagcccggccagcccccccagctgctgatctacgccgcctccaccctgcactccggcatccccgacaggttctccggctccggctccggcaccgacttcaccctgaagatctccagggtggaggccgaggacgtgggcgtgtactactgccagcagtccaaggaggaccccaggaccttcggccagggcaccaagctggagatcaagggaggcggtggatcaggcggaggtggctcaggtggaggcggttctgaggtgcagctggtgcagtccggcgccgaggtgaagaagcccggcgcctccgtgaaggtgtcctgcaaggcctccggctacaccttcaccgactacaacatggactgggtgaggcaggcccccggccagggcctggagtggatgggcgacatcaaccccaacaacggcggcaccctgtacaaccagaagttcaggggcagggtgaccatgaccgtggacacctccatctccaccgcctacatggagctgtccaggctgaggtccgacgacaccgccgtgtactactgcgccaggtccgaggtgttctacggcaactacgccgactactggggccagggcaccaccgtgaccgtgtcctccgagcccaagtcctgcgacaagacccacacctgccccccctgccccgcccccgaggccgccggcggcccctccgtgttcctgttcccccccaagcccaaggacaccctgatgatctccaggacccccgaggtgacctgcgtggtggtggacgtgtcccacgaggaccccgaggtgaagttcaactggtacgtggacggcgtggaggtgcacaacgccaagaccaagcccagggaggagcagtacaactccacctacagggtggtgtccgtgctgaccgtgctgcaccaggactggctgaacggcaaggagtacaagtgcaaggtgtccaacaaggccctgcccgcccccatcgagaagaccatctccaaggccaagggccagcccagggagccccaggtgtgcaccctgcccccctccagggacgagctgaccaagaaccaggtgtccctgtcctgcgccgtgaagggcttctacccctccgacatcgccgtggagtgggagtccaacggccagcccgagaacaactacaagaccaccccccccgtgctggactccgacggctccttcttcctggtgtccaagctgaccgtggacaagtccaggtggcagcagggcaacgtgttctcctgctccgtgatgcacgaggccctgcacaaccactacacccagaagtccctgtccctgtcccccggcaagtaa

SEQ ID NO: 83 - DNA, 1437 bp, Artificial Sequence
  83
gacatcgtgctgacccagacccccctgtccctgtccgtgacccccggccagcccgcctccatctcctgcaaggcctcccagtccgtggactacgacggcgactcctacatgaactggtacctgcagaagcccggccagcccccccagctgctgatctacgccgcctccaccctgcactccggcatccccgacaggttctccggctccggctccggcaccgacttcaccctgaagatctccagggtggaggccgaggacgtgggcgtgtactactgccagcagtccaaggaggaccccaggaccttcggccagggcaccaagctggagatcaagggaggcggtggatcaggcggaggtggctcaggtggaggcggttctgaggtgcagctggtgcagtccggcgccgaggtgaagaagcccggcgcctccgtgaaggtgtcctgcaaggcctccggctacaccttcaccgactacaacatggactgggtgaggcaggcccccggccagggcctggagtggatcggcgacatcaaccccaacaacggcggcaccctgtacaaccagaagttcaggggcagggtgaccctgaccgtggacacctccatctccaccgcctacatggagctgtccaggctgaggtccgacgacaccgccgtgtactactgcgccaggtccgaggtgttctacggcaactacgccgactactggggccagggcaccaccgtgaccgtgtcctccgagcccaagtcctgcgacaagacccacacctgccccccctgccccgcccccgaggccgccggcggcccctccgtgttcctgttcccccccaagcccaaggacaccctgatgatctccaggacccccgaggtgacctgcgtggtggtggacgtgtcccacgaggaccccgaggtgaagttcaactggtacgtggacggcgtggaggtgcacaacgccaagaccaagcccagggaggagcagtacaactccacctacagggtggtgtccgtgctgaccgtgctgcaccaggactggctgaacggcaaggagtacaagtgcaaggtgtccaacaaggccctgcccgcccccatcgagaagaccatctccaaggccaagggccagcccagggagccccaggtgtgcaccctgcccccctccagggacgagctgaccaagaaccaggtgtccctgtcctgcgccgtgaagggcttctacccctccgacatcgccgtggagtgggagtccaacggccagcccgagaacaactacaagaccaccccccccgtgctggactccgacggctccttcttcctggtgtccaagctgaccgtggacaagtccaggtggcagcagggcaacgtgttctcctgctccgtgatgcacgaggccctgcacaaccactacacccagaagtccctgtccctgtcccccggcaagtaa

SEQ ID NO: 84 - DNA, 1437 bp, Artificial Sequence
  84
gacatcgtgctgacccagacccccctgtccctgtccgtgacccccggccagcccgcctccatctcctgcaaggcctcccagtccgtggactacgacggcgactcctacatgaactggtacctgcagaagcccggccagcccccccagctgctgatctacgccgcctccaccctgcactccggcatccccgacaggttctccggctccggctccggcaccgacttcaccctgaagatctccagggtggaggccgaggacgtgggcgtgtactactgccagcagtccaaggaggaccccaggaccttcggccagggcaccaagctggagatcaagggaggcggtggatcaggcggaggtggctcaggtggaggcggttctgaggtgcagctggtgcagtccggcgccgaggtgaagaagcccggcgcctccgtgaaggtgtcctgcaaggcctccggctacaccttcaccgactacaacatggactgggtgaggcaggcccccggccagggcctggagtggatcggcgacatcaaccccaacaacggcggcaccctgtacaaccagaagttcaggggcagggtgaccctgaccgtggacaagtccatctccaccgcctacatggagctgtccaggctgaggtccgacgacaccgccgtgtactactgcgccaggtccgaggtgttctacggcaactacgccgactactggggccagggcaccaccgtgaccgtgtcctccgagcccaagtcctgcgacaagacccacacctgccccccctgccccgcccccgaggccgccggcggcccctccgtgttcctgttcccccccaagcccaaggacaccctgatgatctccaggacccccgaggtgacctgcgtggtggtggacgtgtcccacgaggaccccgaggtgaagttcaactggtacgtggacggcgtggaggtgcacaacgccaagaccaagcccagggaggagcagtacaactccacctacagggtggtgtccgtgctgaccgtgctgcaccaggactggctgaacggcaaggagtacaagtgcaaggtgtccaacaaggccctgcccgcccccatcgagaagaccatctccaaggccaagggccagcccagggagccccaggtgtgcaccctgcccccctccagggacgagctgaccaagaaccaggtgtccctgtcctgcgccgtgaagggcttctacccctccgacatcgccgtggagtgggagtccaacggccagcccgagaacaactacaagaccaccccccccgtgctggactccgacggctccttcttcctggtgtccaagctgaccgtggacaagtccaggtggcagcagggcaacgtgttctcctgctccgtgatgcacgaggccctgcacaaccactacacccagaagtccctgtccctgtcccccggcaagtaa

SEQ ID NO: 85 - DNA, 1437 bp, Artificial Sequence
  85
gacatcgtgctgacccagacccccctgtccctgtccgtgacccccggccagcccgcctccatctcctgcaaggcctcccagtccgtggactacgacggcgactcctacatgaactggtacctgcagaagcccggccagcccccccagctgctgatctacgccgcctccaccctgcactccggcatccccgacaggttctccggctccggctccggcaccgacttcaccctgaagatctccagggtggaggccgaggacgtgggcgtgtactactgccagcagtccaaggaggaccccaggaccttcggccagggcaccaagctggagatcaagggaggcggtggatcaggcggaggtggctcaggtggaggcggttctgaggtgcagctggtgcagtccggcgccgaggtgaagaagcccggcgcctccgtgaaggtgtcctgcaaggcctccggctacaccttcaccgactacaacatggactgggtgaggcaggcccccggcaagggcctggagtggatcggcgacatcaaccccaacaacggcggcaccctgtacaaccagaagttcaggggcagggtgaccctgaccgtggacaagtccatctccaccgcctacatggagctgtccaggctgaggtccgacgacaccgccgtgtactactgcgccaggtccgaggtgttctacggcaactacgccgactactggggccagggcaccaccgtgaccgtgtcctccgagcccaagtcctgcgacaagacccacacctgccccccctgccccgcccccgaggccgccggcggcccctccgtgttcctgttcccccccaagcccaaggacaccctgatgatctccaggacccccgaggtgacctgcgtggtggtggacgtgtcccacgaggaccccgaggtgaagttcaactggtacgtggacggcgtggaggtgcacaacgccaagaccaagcccagggaggagcagtacaactccacctacagggtggtgtccgtgctgaccgtgctgcaccaggactggctgaacggcaaggagtacaagtgcaaggtgtccaacaaggccctgcccgcccccatcgagaagaccatctccaaggccaagggccagcccagggagccccaggtgtgcaccctgcccccctccagggacgagctgaccaagaaccaggtgtccctgtcctgcgccgtgaagggcttctacccctccgacatcgccgtggagtgggagtccaacggccagcccgagaacaactacaagaccaccccccccgtgctggactccgacggctccttcttcctggtgtccaagctgaccgtggacaagtccaggtggcagcagggcaacgtgttctcctgctccgtgatgcacgaggccctgcacaaccactacacccagaagtccctgtccctgtcccccggcaagtaa

SEQ ID NO: 86 - DNA, 1437 bp, Artificial Sequence
  86
gacatcgtgctgacccagtcccccgtgtccctggccgtgcccctgggccagagggccaccatctcctgcaaggcctcccagtccgtggactacgacggcgactcctacatgaactggtaccagcagaagcccggccagccccccaagctgctgatctacgccgcctccaccctgcactccggcatccccgtgaggttctccggctccggctccggcaccgacttcaccctgaacatccaccccgtggaggaggaggacgccgcctcctactactgccagcagtccaaggaggaccccaggaccttcggcggcggcaccaagctggagatcaagggaggcggtggatcaggcggaggtggctcaggtggaggcggttctgaggtgctgctgcagcagtccggccccgaggtggtgaagcccggcgcctccgtgaagatcacctgcaaggcctccggctacaccttcaccgactacaacatggactgggtgaagcagtcccacggcaagtccctggagtggatcggcgacatcaaccccaacaacgccggcaccctgtacaaccagaagttcaggggcagggtgaccctgatcgtggacaagtcctcctccaccgcctacatggagctgaggtccctgacctccgacgacaccgccgtgtactactgcgccaggtccgaggtgttctacggcaactacgccgactactggggccagggcaccaccctgaccgtgtcctccgagcccaagtcctgcgacaagacccacacctgccccccctgccccgcccccgaggccgccggcggcccctccgtgttcctgttcccccccaagcccaaggacaccctgatgatctccaggacccccgaggtgacctgcgtggtggtggacgtgtcccacgaggaccccgaggtgaagttcaactggtacgtggacggcgtggaggtgcacaacgccaagaccaagcccagggaggagcagtacaactccacctacagggtggtgtccgtgctgaccgtgctgcaccaggactggctgaacggcaaggagtacaagtgcaaggtgtccaacaaggccctgcccgcccccatcgagaagaccatctccaaggccaagggccagcccagggagccccaggtgtgcaccctgcccccctccagggacgagctgaccaagaaccaggtgtccctgtcctgcgccgtgaagggcttctacccctccgacatcgccgtggagtgggagtccaacggccagcccgagaacaactacaagaccaccccccccgtgctggactccgacggctccttcttcctggtgtccaagctgaccgtggacaagtccaggtggcagcagggcaacgtgttctcctgctccgtgatgcacgaggccctgcacaaccactacacccagaagtccctgtccctgtcccccggcaagtaa

SEQ ID NO: 87 - DNA, 1437 bp, Artificial Sequence
  87
gacatcgtgctgacccagtcccccgtgtccctggccgtgcccctgggccagagggccaccatctcctgcaaggcctcccagtccgtggactacgacgccgactcctacatgaactggtaccagcagaagcccggccagccccccaagctgctgatctacgccgcctccaccctgcactccggcatccccgtgaggttctccggctccggctccggcaccgacttcaccctgaacatccaccccgtggaggaggaggacgccgcctcctactactgccagcagtccaaggaggaccccaggaccttcggcggcggcaccaagctggagatcaagggaggcggtggatcaggcggaggtggctcaggtggaggcggttctgaggtgctgctgcagcagtccggccccgaggtggtgaagcccggcgcctccgtgaagatcacctgcaaggcctccggctacaccttcaccgactacaacatggactgggtgaagcagtcccacggcaagtccctggagtggatcggcgacatcaaccccaacaacggcggcaccctgtacaaccagaagttcaggggcagggtgaccctgatcgtggacaagtcctcctccaccgcctacatggagctgaggtccctgacctccgacgacaccgccgtgtactactgcgccaggtccgaggtgttctacggcaactacgccgactactggggccagggcaccaccctgaccgtgtcctccgagcccaagtcctgcgacaagacccacacctgccccccctgccccgcccccgaggccgccggcggcccctccgtgttcctgttcccccccaagcccaaggacaccctgatgatctccaggacccccgaggtgacctgcgtggtggtggacgtgtcccacgaggaccccgaggtgaagttcaactggtacgtggacggcgtggaggtgcacaacgccaagaccaagcccagggaggagcagtacaactccacctacagggtggtgtccgtgctgaccgtgctgcaccaggactggctgaacggcaaggagtacaagtgcaaggtgtccaacaaggccctgcccgcccccatcgagaagaccatctccaaggccaagggccagcccagggagccccaggtgtgcaccctgcccccctccagggacgagctgaccaagaaccaggtgtccctgtcctgcgccgtgaagggcttctacccctccgacatcgccgtggagtgggagtccaacggccagcccgagaacaactacaagaccaccccccccgtgctggactccgacggctccttcttcctggtgtccaagctgaccgtggacaagtccaggtggcagcagggcaacgtgttctcctgctccgtgatgcacgaggccctgcacaaccactacacccagaagtccctgtccctgtcccccggcaagtaa

SEQ ID NO: 88 - DNA, 60 bp, Artificial Sequence
  88
atggagaccgacaccctgctgctgtgggtgctgctgctgtgggtgcccggctccaccggc